European Patent Application EP 4 212 166 A1, published July 19, 2023. Title: COMPOSITIONS AND METHODS FOR REDUCING IMMUNE RESPONSES AGAINST CELL THERAPIES. Applicant: Juno Therapeutics, Inc. Application EP, filed August 2, 2022. The sequence listing filed with the application follows.

SEQUENCE LISTING (184 sequences)

SEQ ID NO: 1 - protein, 12 aa, synthetic construct
  REGION 1..12: note = Synthetic
  REGION 1..12: note = IgG4 hinge
ESKYGPPCPPCP

SEQ ID NO: 2 - protein, 27 aa, synthetic construct
  REGION 1..27: note = Synthetic
  REGION 1..27: note = CD28 transmembrane domain
FWVLVVVGGVLACYSLLVTVAFIIFWV

SEQ ID NO: 3 - protein, 42 aa, Homo sapiens
  REGION 1..42: note = 4-1BB costimulatory domain
KRGRKKLLYIFKQPFMRPVQTTQEEDGCSCRFPEEEEGGCEL

SEQ ID NO: 4 - protein, 112 aa, synthetic construct
  REGION 1..112: note = Synthetic
  REGION 1..112: note = CD3-zeta intracellular signaling domain
RVKFSRSADAPAYQQGQNQLYNELNLGRREEYDVLDKRRGRDPEMGGKPRRKNPQEGLYNELQKDKMAEAYSEIGMKGERRRGKGHDGLYQGLSTATKDTYDALHMQALPPR

SEQ ID NO: 5 - protein, 69 aa, synthetic construct
  REGION 1..69: note = Synthetic
  REGION 1..69: note = CD28-4-1BB
FWVLVVVGGVLACYSLLVTVAFIIFWVKRGRKKLLYIFKQPFMRPVQTTQEEDGCSCRFPEEEEGGCEL

SEQ ID NO: 6 - protein, 30 aa, synthetic construct
  REGION 1..30: note = Synthetic
CYSLLVTVAFIIFWVKRGRKKLLYIFKQPF

SEQ ID NO: 7 - protein, 16 aa, synthetic construct
  REGION 1..16: note = Synthetic
VAFIIFWVKRGRKKLL

SEQ ID NO: 8 - protein, 15 aa, synthetic construct
  REGION 1..15: note = Synthetic
AFIIFWVKRGRKKLL

SEQ ID NO: 9 - protein, 15 aa, synthetic construct
  REGION 1..15: note = Synthetic
FWVKRGRKKLLYIFK

SEQ ID NO: 10 - protein, 14 aa, synthetic construct
  REGION 1..14: note = Synthetic
FIIFWVKRGRKKLL

SEQ ID NO: 11 - protein, 13 aa, synthetic construct
  REGION 1..13: note = Synthetic
FIIFWVKRGRKKL

SEQ ID NO: 12 - protein, 13 aa, synthetic construct
  REGION 1..13: note = Synthetic
IIFWVKRGRKKLL

SEQ ID NO: 13 - protein, 32 aa, synthetic construct
  REGION 1..32: note = Synthetic
  REGION 1..32: note = Variant junction region
CYSLLVTVAFIIFWVNNKRGRKKLLYIFKQPF

SEQ ID NO: 14 - protein, 14 aa, synthetic construct
  REGION 1..14: note = Synthetic
  REGION 1..14: note = Variant peptide
IIFWVNNKRGRKKL

SEQ ID NO: 15 - protein, 13 aa, synthetic construct
  REGION 1..13: note = Synthetic
  REGION 1..13: note = Variant peptide
IIFWVNNKRGRKK

SEQ ID NO: 16 - protein, 9 aa, synthetic construct
  REGION 1..9: note = Synthetic
VAFIIFWVK

SEQ ID NO: 17 - protein, 9 aa, synthetic construct
  REGION 1..9: note = Synthetic
AFIIFWVKR

SEQ ID NO: 18 - protein, 9 aa, synthetic construct
  REGION 1..9: note = Synthetic
FIIFWVKRG

SEQ ID NO: 19 - protein, 9 aa, synthetic construct
  REGION 1..9: note = Synthetic
IIFWVKRGR

SEQ ID NO: 20 - protein, 9 aa, synthetic construct
  REGION 1..9: note = Synthetic
IFWVKRGRK

SEQ ID NO: 21 - protein, 9 aa, synthetic construct
  REGION 1..9: note = Synthetic
FWVKRGRKK

SEQ ID NO: 22 - protein, 9 aa, synthetic construct
  REGION 1..9: note = Synthetic
WVKRGRKKL

SEQ ID NO: 23 - protein, 9 aa, synthetic construct
  REGION 1..9: note = Synthetic peptide K28S
VAFIIFWVS

SEQ ID NO: 24 - protein, 9 aa, synthetic construct
  REGION 1..9: note = Synthetic peptide K28S
AFIIFWVSR

SEQ ID NO: 25 - protein, 9 aa, synthetic construct
  REGION 1..9: note = Synthetic peptide K28S
FIIFWVSRG

SEQ ID NO: 26 - protein, 9 aa, synthetic construct
  REGION 1..9: note = Synthetic peptide K28S
IIFWVSRGR

SEQ ID NO: 27 - protein, 9 aa, synthetic construct
  REGION 1..9: note = Synthetic peptide K28S
IFWVSRGRK

SEQ ID NO: 28 - protein, 9 aa, synthetic construct
  REGION 1..9: note = Synthetic peptide K28S
FWVSRGRKK

SEQ ID NO: 29 - protein, 9 aa, synthetic construct
  REGION 1..9: note = Synthetic peptide K28S
WVSRGRKKL

SEQ ID NO: 30 - protein, 9 aa, synthetic construct
  REGION 1..9: note = Synthetic peptide K28L
VAFIIFWVL

SEQ ID NO: 31 - protein, 9 aa, synthetic construct
  REGION 1..9: note = Synthetic peptide K28L
AFIIFWVLR

SEQ ID NO: 32 - protein, 9 aa, synthetic construct
  REGION 1..9: note = Synthetic peptide K28L
FIIFWVLRG

SEQ ID NO: 33 - protein, 9 aa, synthetic construct
  REGION 1..9: note = Synthetic peptide K28L
IIFWVLRGR

SEQ ID NO: 34 - protein, 9 aa, synthetic construct
  REGION 1..9: note = Synthetic peptide K28L
IFWVLRGRK

SEQ ID NO: 35 - protein, 9 aa, synthetic construct
  REGION 1..9: note = Synthetic peptide K28L
FWVLRGRKK

SEQ ID NO: 36 - protein, 9 aa, synthetic construct
  REGION 1..9: note = Synthetic peptide K28L
WVLRGRKKL

SEQ ID NO: 37 - protein, 9 aa, synthetic construct
  REGION 1..9: note = Synthetic peptide K28H
VAFIIFWVH

SEQ ID NO: 38 - protein, 9 aa, synthetic construct
  REGION 1..9: note = Synthetic peptide K28H
AFIIFWVHR

SEQ ID NO: 39 - protein, 9 aa, synthetic construct
  REGION 1..9: note = Synthetic peptide K28H
FIIFWVHRG

SEQ ID NO: 40 - protein, 9 aa, synthetic construct
  REGION 1..9: note = Synthetic peptide K28H
IIFWVHRGR

SEQ ID NO: 41 - protein, 9 aa, synthetic construct
  REGION 1..9: note = Synthetic peptide K28H
IFWVHRGRK

SEQ ID NO: 42 - protein, 9 aa, synthetic construct
  REGION 1..9: note = Synthetic peptide K28H
FWVHRGRKK

SEQ ID NO: 43 - protein, 9 aa, synthetic construct
  REGION 1..9: note = Synthetic peptide K28H
WVHRGRKKL

SEQ ID NO: 44 - protein, 9 aa, synthetic construct
  REGION 1..9: note = Synthetic peptide K28A
VAFIIFWVA

SEQ ID NO: 45 - protein, 9 aa, synthetic construct
  REGION 1..9: note = Synthetic peptide K28A
AFIIFWVAR

SEQ ID NO: 46 - protein, 9 aa, synthetic construct
  REGION 1..9: note = Synthetic peptide K28A
IIFWVARGR

SEQ ID NO: 47 - protein, 9 aa, synthetic construct
  REGION 1..9: note = Synthetic peptide K28A
IFWVARGRK

SEQ ID NO: 48 - protein, 9 aa, synthetic construct
  REGION 1..9: note = Synthetic peptide K28A
FWVARGRKK

SEQ ID NO: 49 - protein, 9 aa, synthetic construct
  REGION 1..9: note = Synthetic peptide K28A
WVARGRKKL

SEQ ID NO: 50 - protein, 9 aa, synthetic construct
  REGION 1..9: note = Synthetic peptide K28Q
VAFIIFWVQ

SEQ ID NO: 51 - protein, 9 aa, synthetic construct
  REGION 1..9: note = Synthetic peptide K28Q
AFIIFWVQR

SEQ ID NO: 52 - protein, 9 aa, synthetic construct
  REGION 1..9: note = Synthetic peptide K28Q
FIIFWVQRG

SEQ ID NO: 53 - protein, 9 aa, synthetic construct
  REGION 1..9: note = Synthetic peptide K28Q
IIFWVQRGR

SEQ ID NO: 54 - protein, 9 aa, synthetic construct
  REGION 1..9: note = Synthetic peptide K28Q
IFWVQRGRK

SEQ ID NO: 55 - protein, 9 aa, synthetic construct
  REGION 1..9: note = Synthetic peptide K28Q
FWVQRGRKK

SEQ ID NO: 56 - protein, 9 aa, synthetic construct
  REGION 1..9: note = Synthetic peptide K28Q
WVQRGRKKL

SEQ ID NO: 57 - protein, 9 aa, synthetic construct
  REGION 1..9: note = Synthetic peptide R31S
IIFWVKRGS

SEQ ID NO: 58 - protein, 9 aa, synthetic construct
  REGION 1..9: note = Synthetic peptide R31S
IFWVKRGSK

SEQ ID NO: 59 - protein, 9 aa, synthetic construct
  REGION 1..9: note = Synthetic peptide R31S
FWVKRGSKK

SEQ ID NO: 60 - protein, 9 aa, synthetic construct
  REGION 1..9: note = Synthetic peptide R31S
WVKRGSKKL

SEQ ID NO: 61 - protein, 9 aa, synthetic construct
  REGION 1..9: note = Synthetic peptide R31L
IIFWVKRGL

SEQ ID NO: 62 - protein, 9 aa, synthetic construct
  REGION 1..9: note = Synthetic peptide R31L
IFWVKRGLK

SEQ ID NO: 63 - protein, 9 aa, synthetic construct
  REGION 1..9: note = Synthetic peptide R31L
FWVKRGLKK

SEQ ID NO: 64 - protein, 9 aa, synthetic construct
  REGION 1..9: note = Synthetic peptide R31L
WVKRGLKKL

SEQ ID NO: 65 - protein, 9 aa, synthetic construct
  REGION 1..9: note = Synthetic peptide R31H
IIFWVKRGH

SEQ ID NO: 66 - protein, 9 aa, synthetic construct
  REGION 1..9: note = Synthetic peptide R31H
IFWVKRGHK

SEQ ID NO: 67 - protein, 9 aa, synthetic construct
  REGION 1..9: note = Synthetic peptide R31H
FWVKRGHKK

SEQ ID NO: 68 - protein, 9 aa, synthetic construct
  REGION 1..9: note = Synthetic peptide R31H
WVKRGHKKL

SEQ ID NO: 69 - protein, 9 aa, synthetic construct
  REGION 1..9: note = Synthetic peptide R31A
IIFWVKRGA

SEQ ID NO: 70 - protein, 9 aa, synthetic construct
  REGION 1..9: note = Synthetic peptide R31A
IFWVKRGAK

SEQ ID NO: 71 - protein, 9 aa, synthetic construct
  REGION 1..9: note = Synthetic peptide R31A
FWVKRGAKK

SEQ ID NO: 72 - protein, 9 aa, synthetic construct
  REGION 1..9: note = Synthetic peptide R31A
WVKRGAKKL

SEQ ID NO: 73 - protein, 9 aa, synthetic construct
  REGION 1..9: note = Synthetic peptide R31N
IIFWVKRGN

SEQ ID NO: 74 - protein, 9 aa, synthetic construct
  REGION 1..9: note = Synthetic peptide R31N
IFWVKRGNK

SEQ ID NO: 75 - protein, 9 aa, synthetic construct
  REGION 1..9: note = Synthetic peptide R31N
FWVKRGNKK

SEQ ID NO: 76 - protein, 9 aa, synthetic construct
  REGION 1..9: note = Synthetic peptide R31N
WVKRGNKKL

SEQ ID NO: 77 - protein, 9 aa, synthetic construct
  REGION 1..9: note = Synthetic peptide K28Q/R31S
IIFWVQRGS

SEQ ID NO: 78 - protein, 9 aa, synthetic construct
  REGION 1..9: note = Synthetic peptide K28Q/R31S
IFWVQRGSK

SEQ ID NO: 79 - protein, 9 aa, synthetic construct
  REGION 1..9: note = Synthetic peptide K28Q/R31S
FWVQRGSKK

SEQ ID NO: 80 - protein, 9 aa, synthetic construct
  REGION 1..9: note = Synthetic peptide K28Q/R31S
WVQRGSKKL

SEQ ID NO: 81 - protein, 9 aa, synthetic construct
  REGION 1..9: note = Synthetic peptide K28Q/R31A
IIFWVQRGA

SEQ ID NO: 82 - protein, 9 aa, synthetic construct
  REGION 1..9: note = Synthetic peptide K28Q/R31A
IFWVQRGAK

SEQ ID NO: 83 - protein, 9 aa, synthetic construct
  REGION 1..9: note = Synthetic peptide K28Q/R31A
FWVQRGAKK

SEQ ID NO: 84 - protein, 9 aa, synthetic construct
  REGION 1..9: note = Synthetic peptide K28Q/R31A
WVQRGAKKL

SEQ ID NO: 85 - protein, 9 aa, synthetic construct
  REGION 1..9: note = Synthetic peptide K28Q/R31N
IIFWVQRGN

SEQ ID NO: 86 - protein, 9 aa, synthetic construct
  REGION 1..9: note = Synthetic peptide K28Q/R31N
IFWVQRGNK

SEQ ID NO: 87 - protein, 9 aa, synthetic construct
  REGION 1..9: note = Synthetic peptide K28Q/R31N
FWVQRGNKK

SEQ ID NO: 88 - protein, 9 aa, synthetic construct
  REGION 1..9: note = Synthetic peptide K28Q/R31N
WVQRGNKKL

SEQ ID NO: 89 - protein, 9 aa, synthetic construct
  REGION 1..9: note = Synthetic peptide L34S
WVKRGRKKS

SEQ ID NO: 90 - protein, 9 aa, synthetic construct
  REGION 1..9: note = Synthetic peptide L34A
WVKRGRKKA

SEQ ID NO: 91 - protein, 9 aa, synthetic construct
  REGION 1..9: note = Synthetic peptide K28Q/L34S
WVQRGNKKS

SEQ ID NO: 92 - protein, 9 aa, synthetic construct
  REGION 1..9: note = Synthetic peptide K28Q/L34A
WVQRGNKKA

SEQ ID NO: 93 - protein, 255 aa, synthetic construct
  REGION 1..255: note = Synthetic
  REGION 1..255: note = 4-1BB
MGNSCYNIVATLLLVLNFERTRSLQDPCSNCPAGTFCDNNRNQICSPCPPNSFSSAGGQRTCDICRQCKGVFRTRKECSSTSNAECDCTPGFHCLGAGCSMCEQDCKQGQELTKKGCKDCCFGTFNDQKRGICRPWTNCSLDGKSVLVNGTKERDVVCGPSPADLSPGASSVTPPAPAREPGHSPQIISFFLALTSTALLFLLFFLTLRFSVVKRGRKKLLYIFKQPFMRPVQTTQEEDGCSCRFPEEEEGGCEL

SEQ ID NO: 94 - protein, 220 aa, synthetic construct
  REGION 1..220: note = Synthetic
  REGION 1..220: note = CD28
MLRLLLALNLFPSIQVTGNKILVKQSPMLVAYDNAVNLSCKYSYNLFSREFRASLHKGLDSAVEVCVVYGNYSQQLQVYSKTGFNCDGKLGNESVTFYLQNLYVNQTDIYFCKIEVMYPPPYLDNEKSNGTIIHVKGKHLCPSPLFPGPSKPFWVLVVVGGVLACYSLLVTVAFIIFWVRSKRSRLLHSDYMNMTPRRPGPTRKHYQPYAPPRDFAAYRS

SEQ ID NO: 95 - protein, 164 aa, synthetic construct
  REGION 1..164: note = Synthetic
  REGION 1..164: note = CD3 zeta chain
MKWKALFTAAILQAQLPITEAQSFGLLDPKLCYLLDGILFIYGVILTALFLRVKFSRSADAPAYQQGQNQLYNELNLGRREEYDVLDKRRGRDPEMGGKPQRRKNPQEGLYNELQKDKMAEAYSEIGMKGERRRGKGHDGLYQGLSTATKDTYDALHMQALPPR

SEQ ID NO: 96 - protein, 14 aa, synthetic construct
  REGION 1..14: note = Synthetic
FIIFWVNNKRGRKK

SEQ ID NO: 97 - protein, 14 aa, synthetic construct
  REGION 1..14: note = Synthetic
IFWVNNKRGRKKLL

SEQ ID NO: 98 - protein, 14 aa, synthetic construct
  REGION 1..14: note = Synthetic
FIIFWVNNKRGRKK

SEQ ID NO: 99 - protein, 14 aa, synthetic construct
  REGION 1..14: note = Synthetic
IFWVNNKRGRKKLL

SEQ ID NO: 100 - protein, 9 aa, synthetic construct
  REGION 1..9: note = Synthetic peptide K28R
VAFIIFWVR

SEQ ID NO: 101 - protein, 9 aa, synthetic construct
  REGION 1..9: note = Synthetic peptide K28R
AFIIFWVRR

SEQ ID NO: 102 - protein, 9 aa, synthetic construct
  REGION 1..9: note = Synthetic peptide K28A
FIIFWVARG

SEQ ID NO: 103 - protein, 28 aa, Homo sapiens
  REGION 1..28: note = CD28 transmembrane domain
MFWVLVVVGGVLACYSLLVTVAFIIFWV

SEQ ID NO: 104 - protein, 66 aa, Homo sapiens
  REGION 1..66: note = CD28, including transmembrane
IEVMYPPPYLDNEKSNGTIIHVKGKHLCPSPLFPGPSKPFWVLVVVGGVLACYSLLVTVAFIIFWV

SEQ ID NO: 105 - protein, 112 aa, Homo sapiens
  REGION 1..112: note = CD3 zeta
RVKFSRSAEPPAYQQGQNQLYNELNLGRREEYDVLDKRRGRDPEMGGKPRRKNPQEGLYNELQKDKMAEAYSEIGMKGERRRGKGHDGLYQGLSTATKDTYDALHMQALPPR

SEQ ID NO: 106 - DNA, 36 bp, Homo sapiens
  misc_feature 1..36: note = spacer (IgG4hinge)
  source 1..36: mol_type = unassigned DNA
gaatctaagtacggaccgccctgccccccttgccct

SEQ ID NO: 107 - protein, 119 aa, Homo sapiens
  REGION 1..119: note = Hinge-CH3 spacer
ESKYGPPCPPCPGQPREPQVYTLPPSQEEMTKNQVSLTCLVKGFYPSDIAVEWESNGQPENNYKTTPPVLDSDGSFFLYSRLTVDKSRWQEGNVFSCSVMHEALHNHYTQKSLSLSLGK

SEQ ID NO: 108 - protein, 229 aa, Homo sapiens
  REGION 1..229: note = Hinge-CH2-CH3 spacer
ESKYGPPCPPCPAPEFLGGPSVFLFPPKPKDTLMISRTPEVTCVVVDVSQEDPEVQFNWYVDGVEVHNAKTKPREEQFNSTYRVVSVLTVLHQDWLNGKEYKCKVSNKGLPSSIEKTISKAKGQPREPQVYTLPPSQEEMTKNQVSLTCLVKGFYPSDIAVEWESNGQPENNYKTTPPVLDSDGSFFLYSRLTVDKSRWQEGNVFSCSVMHEALHNHYTQKSLSLSLGK

SEQ ID NO: 109 - protein, 282 aa, Homo sapiens
  REGION 1..282: note = IgD-hinge-Fc
RWPESPKAQASSVPTAQPQAEGSLAKATTAPATTRNTGRGGEEKKKEKEKEEQEERETKTPECPSHTQPLGVYLLTPAVQDLWLRDKATFTCFVVGSDLKDAHLTWEVAGKVPTGGVEEGLLERHSNGSQSQHSRLTLPRSLWNAGTSVTCTLNHPSLPPQRLMALREPAAQAPVKLSLNLLASSDPPEAASWLLCEVSGFSPPNILLMWLEDQREVNTSGFAPARPPPQPGSTTFWAWSVLRVPAPPSPQPATYTCVVSHEDSRTLLNASRSLEVSYVTDH

SEQ ID NO: 110 - protein, 24 aa, synthetic construct
  REGION 1..24: note = Synthetic
  REGION 1..24: note = T2A
LEGGGEGRGSLLTCGDVEENPGPR

SEQ ID NO: 111 - protein, 357 aa, synthetic construct
  REGION 1..357: note = Synthetic
  REGION 1..357: note = tEGFR
MLLLVTSLLLCELPHPAFLLIPRKVCNGIGIGEFKDSLSINATNIKHFKNCTSISGDLHILPVAFRGDSFTHTPPLDPQELDILKTVKEITGFLLIQAWPENRTDLHAFENLEIIRGRTKQHGQFSLAVVSLNITSLGLRSLKEISDGDVIISGNKNLCYANTINWKKLFGTSGQKTKIISNRGENSCKATGQVCHALCSPEGCWGPEPRDCVSCRNVSRGRECVDKCNLLEGEPREFVENSECIQCHPECLPQAMNITCTGRGPDNCIQCAHYIDGPHCVKTCPAGVMGENNTLVWKYADAGHVCHLCHPNCTYGCTGPGLEGCPTNGPKIPSIATGMVGALLLLLVVALGIGLFM

SEQ ID NO: 112 - protein, 41 aa, Homo sapiens
  REGION 1..41: note = CD28 cytoplasmic domain
RSKRSRLLHSDYMNMTPRRPGPTRKHYQPYAPPRDFAAYRS

SEQ ID NO: 113 - protein, 41 aa, Homo sapiens
  REGION 1..41: note = CD28 cytoplasmic domain
RSKRSRGGHSDYMNMTPRRPGPTRKHYQPYAPPRDFAAYRS

SEQ ID NO: 114 - protein, 69 aa, synthetic construct
  REGION 1..69: note = Synthetic K28A
FWVLVVVGGVLACYSLLVTVAFIIFWVARGRKKLLYIFKQPFMRPVQTTQEEDGCSCRFPEEEEGGCEL

SEQ ID NO: 115 - protein, 69 aa, synthetic construct
  REGION 1..69: note = Synthetic K28H
FWVLVVVGGVLACYSLLVTVAFIIFWVHRGRKKLLYIFKQPFMRPVQTTQEEDGCSCRFPEEEEGGCEL

SEQ ID NO: 116 - protein, 69 aa, synthetic construct
  REGION 1..69: note = Synthetic K28L
FWVLVVVGGVLACYSLLVTVAFIIFWVLRGRKKLLYIFKQPFMRPVQTTQEEDGCSCRFPEEEEGGCEL

SEQ ID NO: 117 - protein, 69 aa, synthetic construct
  REGION 1..69: note = Synthetic K28Q
FWVLVVVGGVLACYSLLVTVAFIIFWVQRGRKKLLYIFKQPFMRPVQTTQEEDGCSCRFPEEEEGGCEL

SEQ ID NO: 118 - protein, 69 aa, synthetic construct
  REGION 1..69: note = Synthetic K28S
FWVLVVVGGVLACYSLLVTVAFIIFWVSRGRKKLLYIFKQPFMRPVQTTQEEDGCSCRFPEEEEGGCEL

SEQ ID NO: 119 - protein, 69 aa, synthetic construct
  REGION 1..69: note = Synthetic R31A
FWVLVVVGGVLACYSLLVTVAFIIFWVKRGAKKLLYIFKQPFMRPVQTTQEEDGCSCRFPEEEEGGCEL

SEQ ID NO: 120 - protein, 69 aa, synthetic construct
  REGION 1..69: note = Synthetic R31H
FWVLVVVGGVLACYSLLVTVAFIIFWVKRGHKKLLYIFKQPFMRPVQTTQEEDGCSCRFPEEEEGGCEL

SEQ ID NO: 121 - protein, 69 aa, synthetic construct
  REGION 1..69: note = Synthetic R31L
FWVLVVVGGVLACYSLLVTVAFIIFWVKRGLKKLLYIFKQPFMRPVQTTQEEDGCSCRFPEEEEGGCEL

SEQ ID NO: 122 - protein, 69 aa, synthetic construct
  REGION 1..69: note = Synthetic R31N
FWVLVVVGGVLACYSLLVTVAFIIFWVKRGNKKLLYIFKQPFMRPVQTTQEEDGCSCRFPEEEEGGCEL

SEQ ID NO: 123 - protein, 69 aa, synthetic construct
  REGION 1..69: note = Synthetic L34A
FWVLVVVGGVLACYSLLVTVAFIIFWVKRGRKKALYIFKQPFMRPVQTTQEEDGCSCRFPEEEEGGCEL

SEQ ID NO: 124 - protein, 69 aa, synthetic construct
  REGION 1..69: note = Synthetic L34S
FWVLVVVGGVLACYSLLVTVAFIIFWVKRGRKKSLYIFKQPFMRPVQTTQEEDGCSCRFPEEEEGGCEL

SEQ ID NO: 125 - protein, 69 aa, synthetic construct
  REGION 1..69: note = Synthetic K28Q/R31A
FWVLVVVGGVLACYSLLVTVAFIIFWVQRGAKKLLYIFKQPFMRPVQTTQEEDGCSCRFPEEEEGGCEL

SEQ ID NO: 126 - protein, 69 aa, synthetic construct
  REGION 1..69: note = Synthetic K28Q/R31N
FWVLVVVGGVLACYSLLVTVAFIIFWVQRGNKKLLYIFKQPFMRPVQTTQEEDGCSCRFPEEEEGGCEL

SEQ ID NO: 127 - protein, 69 aa, synthetic construct
  REGION 1..69: note = Synthetic K28Q/R31S
FWVLVVVGGVLACYSLLVTVAFIIFWVQRGSKKLLYIFKQPFMRPVQTTQEEDGCSCRFPEEEEGGCEL

SEQ ID NO: 128 - protein, 69 aa, synthetic construct
  REGION 1..69: note = Synthetic K28Q/L34A
FWVLVVVGGVLACYSLLVTVAFIIFWVQRGRKKALYIFKQPFMRPVQTTQEEDGCSCRFPEEEEGGCEL

SEQ ID NO: 129 - protein, 69 aa, synthetic construct
  REGION 1..69: note = Synthetic K28Q/L34A
FWVLVVVGGVLACYSLLVTVAFIIFWVQRGRKKSLYIFKQPFMRPVQTTQEEDGCSCRFPEEEEGGCEL

SEQ ID NO: 130 - protein, 69 aa, synthetic construct
  REGION 1..69: note = Synthetic R31N/L34A
FWVLVVVGGVLACYSLLVTVAFIIFWVKRGNKKALYIFKQPFMRPVQTTQEEDGCSCRFPEEEEGGCEL

SEQ ID NO: 131 - protein, 69 aa, synthetic construct
  REGION 1..69: note = Synthetic R31N/L34S
FWVLVVVGGVLACYSLLVTVAFIIFWVKRGNKKSLYIFKQPFMRPVQTTQEEDGCSCRFPEEEEGGCEL

SEQ ID NO: 132 - protein, 69 aa, synthetic construct
  REGION 1..69: note = Synthetic K28Q/R31N/L34A
FWVLVVVGGVLACYSLLVTVAFIIFWVQRGNKKALYIFKQPFMRPVQTTQEEDGCSCRFPEEEEGGCEL

SEQ ID NO: 133 - protein, 69 aa, synthetic construct
  REGION 1..69: note = Synthetic K28Q/R31N/L34S
FWVLVVVGGVLACYSLLVTVAFIIFWVQRGNKKSLYIFKQPFMRPVQTTQEEDGCSCRFPEEEEGGCEL

SEQ ID NO: 134 - protein, 71 aa, synthetic construct
  REGION 1..71: note = Synthetic
  REGION 1..71: note = NN Insertion
FWVLVVVGGVLACYSLLVTVAFIIFWVNNKRGRKKLLYIFKQPFMRPVQTTQEEDGCSCRFPEEEEGGCEL

SEQ ID NO: 135 - protein, 70 aa, synthetic construct
  REGION 1..70: note = Synthetic
MFWVLVVVGGVLACYSLLVTVAFIIFWVKRGRKKLLYIFKQPFMRPVQTTQEEDGCSCRFPEEEEGGCEL

SEQ ID NO: 136 - protein, 108 aa, synthetic construct
  REGION 1..108: note = Synthetic
IEVMYPPPYLDNEKSNGTIIHVKGKHLCPSPLFPGPSKPFWVLVVVGGVLACYSLLVTVAFIIFWVKRGRKKLLYIFKQPFMRPVQTTQEEDGCSCRFPEEEEGGCEL

SEQ ID NO: 137 - protein, 26 aa, synthetic construct
  REGION 1..26: note = Synthetic
  REGION 1..26: note = junction region
SLLVTVAFIIFWVKRGRKKLLYIFKQ

SEQ ID NO: 138 - protein, 26 aa, synthetic construct
  REGION 1..26: note = Synthetic
  REGION 1..26: note = junction region K14A
SLLVTVAFIIFWVARGRKKLLYIFKQ

SEQ ID NO: 139 - protein, 26 aa, synthetic construct
  REGION 1..26: note = Synthetic
  REGION 1..26: note = junction region K14H
SLLVTVAFIIFWVHRGRKKLLYIFKQ

SEQ ID NO: 140 - protein, 26 aa, synthetic construct
  REGION 1..26: note = Synthetic
  REGION 1..26: note = junction region K14L
SLLVTVAFIIFWVLRGRKKLLYIFKQ

SEQ ID NO: 141 - protein, 26 aa, synthetic construct
  REGION 1..26: note = Synthetic
  REGION 1..26: note = junction region K14Q
SLLVTVAFIIFWVQRGRKKLLYIFKQ

SEQ ID NO: 142 - protein, 26 aa, synthetic construct
  REGION 1..26: note = Synthetic
  REGION 1..26: note = junction region K14S
SLLVTVAFIIFWVSRGRKKLLYIFKQ

SEQ ID NO: 143 - protein, 26 aa, synthetic construct
  REGION 1..26: note = Synthetic
  REGION 1..26: note = junction region R17A
SLLVTVAFIIFWVKRGAKKLLYIFKQ

SEQ ID NO: 144 - protein, 26 aa, synthetic construct
  REGION 1..26: note = Synthetic
  REGION 1..26: note = junction region R17H
SLLVTVAFIIFWVKRGHKKLLYIFKQ

SEQ ID NO: 145 - protein, 26 aa, synthetic construct
  REGION 1..26: note = Synthetic
  REGION 1..26: note = junction region R17H
SLLVTVAFIIFWVKRGLKKLLYIFKQ

SEQ ID NO: 146 - protein, 26 aa, synthetic construct
  REGION 1..26: note = Synthetic
  REGION 1..26: note = junction region R17N
SLLVTVAFIIFWVKRGNKKLLYIFKQ

SEQ ID NO: 147 - protein, 26 aa, synthetic construct
  REGION 1..26: note = Synthetic
  REGION 1..26: note = junction region L20A
SLLVTVAFIIFWVKRGRKKALYIFKQ

SEQ ID NO: 148 - protein, 26 aa, synthetic construct
  REGION 1..26: note = Synthetic
  REGION 1..26: note = junction region L20S
SLLVTVAFIIFWVKRGRKKSLYIFKQ

SEQ ID NO: 149 - protein, 26 aa, synthetic construct
  REGION 1..26: note = Synthetic
  REGION 1..26: note = junction region K14Q/R17A
SLLVTVAFIIFWVQRGAKKLLYIFKQ

SEQ ID NO: 150 - protein, 26 aa, synthetic construct
  REGION 1..26: note = Synthetic
  REGION 1..26: note = junction region K14Q/R17N
SLLVTVAFIIFWVQRGNKKLLYIFKQ

SEQ ID NO: 151 - protein, 26 aa, synthetic construct
  REGION 1..26: note = Synthetic
  REGION 1..26: note = junction region K14Q/R17S
SLLVTVAFIIFWVQRGSKKLLYIFKQ

SEQ ID NO: 152 - protein, 26 aa, synthetic construct
  REGION 1..26: note = Synthetic
  REGION 1..26: note = junction region K14Q/L20A
SLLVTVAFIIFWVQRGRKKALYIFKQ

SEQ ID NO: 153 - protein, 26 aa, synthetic construct
  REGION 1..26: note = Synthetic
  REGION 1..26: note = junction region K14Q/L20S
SLLVTVAFIIFWVQRGRKKSLYIFKQ

SEQ ID NO: 154 - protein, 26 aa, synthetic construct
  REGION 1..26: note = Synthetic
  REGION 1..26: note = junction region R17N/L20A
SLLVTVAFIIFWVKRGNKKALYIFKQ

SEQ ID NO: 155 - protein, 26 aa, synthetic construct
  REGION 1..26: note = Synthetic
  REGION 1..26: note = junction region R17N/L20S
SLLVTVAFIIFWVKRGNKKSLYIFKQ

SEQ ID NO: 156 - protein, 26 aa, synthetic construct
  REGION 1..26: note = Synthetic
  REGION 1..26: note = junction region K14Q/R17N/L20A
SLLVTVAFIIFWVQRGNKKALYIFKQ

SEQ ID NO: 157 - protein, 26 aa, synthetic construct
  REGION 1..26: note = Synthetic
  REGION 1..26: note = junction region K14Q/R17N/L20S
SLLVTVAFIIFWVQRGNKKSLYIFKQ

SEQ ID NO: 158 - DNA, 36 bp, Homo sapiens; identical to SEQ ID NO: 106
  misc_feature 1..36: note = spacer (IgG4hinge)
  source 1..36: mol_type = unassigned DNA

SEQ ID NO: 159 - protein, 112 aa, synthetic construct
  REGION 1..112: note = Synthetic
  REGION 1..112: note = CD3 Zeta
RVKFSRSADAPAYKQGQNQLYNELNLGRREEYDVLDKRRGRDPEMGGKPRRKNPQEGLYNELQKDKMAEAYSEIGMKGERRRGKGHDGLYQGLSTATKDTYDALHMQALPPR

SEQ ID NO: 160 - protein, 36 aa, synthetic construct
  REGION 1..36: note = Synthetic
CYSLLVTVAFIIFWVKRGRKKLLYIFKQPFMRPVQT

SEQ ID NO: 161 - protein, 15 aa, synthetic construct
  REGION 1..15: note = Synthetic
CYSLLVTVAFIIFWV

SEQ ID NO: 162 - protein, 15 aa, synthetic construct
  REGION 1..15: note = Synthetic
LLVTVAFIIFWVKRG

SEQ ID NO: 163 - protein, 15 aa, synthetic construct
  REGION 1..15: note = Synthetic
TVAFIIFWVKRGRKK

SEQ ID NO: 164 - protein, 15 aa, synthetic construct
  REGION 1..15: note = Synthetic
FIIFWVKRGRKKLLY

SEQ ID NO: 165 - protein, 15 aa, synthetic construct
  REGION 1..15: note = Synthetic
FWVKRGRKKLLYIFK

SEQ ID NO: 166 - protein, 15 aa, synthetic construct
  REGION 1..15: note = Synthetic
KRGRKKLLYIFKQPF

SEQ ID NO: 167 - protein, 15 aa, synthetic construct
  REGION 1..15: note = Synthetic
RKKLLYIFKQPFMRP

SEQ ID NO: 168 - protein, 15 aa, synthetic construct
  REGION 1..15: note = Synthetic
LLYIFKQPFMRPVQT

SEQ ID NO: 169 - protein, 15 aa, synthetic construct
  REGION 1..15: note = Synthetic peptide R31H
TVAFIIFWVKRGHKK

SEQ ID NO: 170 - protein, 15 aa, synthetic construct
  REGION 1..15: note = Synthetic peptide R31H
FIIFWVKRGHKKLLY

SEQ ID NO: 171 - protein, 15 aa, synthetic construct
  REGION 1..15: note = Synthetic peptide R31H
FWVKRGHKKLLYIFK

SEQ ID NO: 172 - protein, 15 aa, synthetic construct
  REGION 1..15: note = Synthetic peptide R31H
KRGHKKLLYIFKQPF

SEQ ID NO: 173 - protein, 15 aa, synthetic construct
  REGION 1..15: note = Synthetic peptide R31H
HKKLLYIFKQPFMRP

SEQ ID NO: 174 - protein, 15 aa, synthetic construct
  REGION 1..15: note = Synthetic peptide R31N
TVAFIIFWVKRGNKK

SEQ ID NO: 175 - protein, 15 aa, synthetic construct
  REGION 1..15: note = Synthetic peptide R31N
FIIFWVKRGNKKLLY

SEQ ID NO: 176 - protein, 15 aa, synthetic construct
  REGION 1..15: note = Synthetic peptide R31N
FWVKRGNKKLLYIFK

SEQ ID NO: 177 - protein, 15 aa, synthetic construct
  REGION 1..15: note = Synthetic peptide R31N
KRGNKKLLYIFKQPF

SEQ ID NO: 178 - protein, 15 aa, synthetic construct
  REGION 1..15: note = Synthetic peptide R31N
NKKLLYIFKQPFMRP

SEQ ID NO: 179 - protein, 15 aa, synthetic construct
  REGION 1..15: note = Synthetic peptide L34A
FIIFWVKRGRKKALY

SEQ ID NO: 180 - protein, 15 aa, synthetic construct
  REGION 1..15: note = Synthetic peptide L34A
FWVKRGRKKALYIFK

SEQ ID NO: 181 - protein, 15 aa, synthetic construct
  REGION 1..15: note = Synthetic peptide L34A
KRGRKKALYIFKQPF

SEQ ID NO: 182 - protein, 15 aa, synthetic construct
  REGION 1..15: note = Synthetic peptide L34A
RKKALYIFKQPFMRP

SEQ ID NO: 183 - protein, 69 aa, synthetic construct
  REGION 1..69: note = Synthetic R31S
FWVLVVVGGVLACYSLLVTVAFIIFWVKRGSKKLLYIFKQPFMRPVQTTQEEDGCSCRFPEEEEGGCEL

SEQ ID NO: 184 - protein, 26 aa, synthetic construct
  REGION 1..26: note = Synthetic
  REGION 1..26: note = junction region K31S
SLLVTVAFIIFWVKRGSKKLLYIFKQ